European Patent Specification EP 3 400 290 B1, published April 5, 2023. Title: VIRUS STRAIN. Applicant: Replimune Limited. The sequence listing filed with the application follows.

SEQUENCE LISTING (45 sequences)

SEQ ID NO: 1 - DNA, 426 bp, Mus musculus
atgtggctgcagaatttacttttcctgggcattgtggtctacagcctctcagcacccacccgctcacccatcactgtcacccggccttggaagcatgtagaggccatcaaagaagccctgaacctcctggatgacatgcctgtcacattgaatgaagaggtagaagtcgtctctaacgagttctccttcaagaagctaacatgtgtgcagacccgcctgaagatattcgagcagggtctacggggcaatttcaccaaactcaagggcgccttgaacatgacagccagctactaccagacatactgccccccaactccggaaacggactgtgaaacacaagttaccacctatgcggatttcatagacagccttaaaacctttctgactgatatcccctttgaatgcaaaaaaccagtccaaaaatga

SEQ ID NO: 2 - DNA, 426 bp, Mus musculus
atgtggctccagaacctcctcttcctcggtatcgtcgtgtattcactctccgcacctactcgctcacctatcactgtcaccagaccctggaagcacgtggaggccatcaaggaggctctgaacctgctggacgatatgccagtgaccctgaacgaggaggtggaggtggtgagcaacgagttctcctttaagaagctgacctgcgtgcagacaaggctgaagatcttcgagcagggcctgagaggaaactttaccaagctgaagggcgccctgaacatgaccgcttcttactaccagacatactgcccccctacccccgagacagactgtgagacacaggtgaccacatacgccgacttcattgatagcctgaaaacattcctgaccgacattccatttgagtgtaagaagcccgtccagaagtaa

SEQ ID NO: 3 - DNA, 435 bp, Homo sapiens
atgtggctgcagagcctgctgctcttgggcactgtggcctgcagcatctctgcacccgcccgctcgcccagccccagcacgcagccctgggagcatgtgaatgccatccaggaggcccggcgtctcctgaacctgagtagagacactgctgctgagatgaatgaaacagtagaagtcatctcagaaatgtttgacctccaggagccgacctgcctacagacccgcctggagctgtacaagcagggcctgcggggcagcctcaccaagctcaagggccccttgaccatgatggccagccactacaagcagcactgccctccaaccccggaaacttcctgtgcaacccagattatcacctttgaaagtttcaaagagaacctgaaggactttctgcttgtcatcccctttgactgctgggagccagtccaggagtga

SEQ ID NO: 4 - DNA, 435 bp, Homo sapiens
atgtggctgcagtccctgctgctgctgggcaccgtcgcctgttctatttccgcacccgcaaggtcaccaagtccatctactcagccttgggagcacgtgaacgcaatccaggaggcacggcggctgctgaacctgagccgggacaccgccgccgagatgaacgagacagtggaagtgatcagcgagatgttcgatctgcaggagcccacctgcctgcagacaaggctggagctgtacaagcagggcctgcgcggctctctgaccaagctgaagggcccactgacaatgatggccagccactataagcagcactgcccccctacccccgagacaagctgtgccacccagatcatcacattcgagtcctttaaggagaacctgaaggattttctgctggtcattccatttgattgttgggagcccgtccaggagtaa

SEQ ID NO: 5 - protein, 141 aa, Mus musculus
MWLQNLLFLGIVVYSLSAPTRSPITVTRPWKHVEAIKEALNLLDDMPVTLNEEVEVVSNEFSFKKLTCVQTRLKIFEQGLRGNFTKLKGALNMTASYYQTYCPPTPETDCETQVTTYADFIDSLKTFLTDIPFECKKPVQK

SEQ ID NO: 6 - protein, 144 aa, Homo sapiens
MWLQSLLLLGTVACSISAPARSPSPSTQPWEHVNAIQEARRLLNLSRDTAAEMNETVEVISEMFDLQEPTCLQTRLELYKQGLRGSLTKLKGPLTMMASHYKQHCPPTPETSCATQIITFESFKENLKDFLLVIPFDCWEPVQE

SEQ ID NO: 7 - DNA, 2010 bp, Gibbon leukemia virus
atggtattgctgcctgggtccatgcttctcacctcaaacctgcaccaccttcggcaccagatgagtcctgggagctggaaaagactgatcatcctcttaagctgcgtattcggcggcggcgggacgagtctgcaaaataagaacccccaccagcccatgaccctcacttggcaggtactgtcccaaactggagacgttgtctgggatacaaaggcagtccagcccccttggacttggtggcccacacttaaacctgatgtatgtgccttggcggctagtcttgagtcctgggatatcccgggaaccgatgtctcgtcctctaaacgagtcagacctccggactcagactatactgccgcttataagcaaatcacctggggagccatagggtgcagctaccctcgggctaggactagaatggcaagctctaccttctacgtatgtccccgggatggccggaccctttcagaagctagaaggtgcggggggctagaatccctatactgtaaagaatgggattgtgagaccacggggaccggttattggctatctaaatcctcaaaagacctcataactgtaaaatgggaccaaaatagcgaatggactcaaaaatttcaacagtgtcaccagaccggctggtgtaacccccttaaaatagatttcacagacaaaggaaaattatccaaggactggataacgggaaaaacctggggattaagattctatgtgtctggacatccaggcgtacagttcaccattcgcttaaaaatcaccaacatgccagctgtggcagtaggtcctgacctcgtccttgtggaacaaggacctcctagaacgtccctcgctctcccacctcctcttcccccaagggaagcgccaccgccatctctccccgactctaactccacagccctggcgactagtgcacaaactcccacggtgagaaaaacaattgttaccctaaacactccgcctcccaccacaggcgacagactttttgatcttgtgcagggggccttcctaaccttaaatgctaccaacccaggggccactgagtcttgctggctttgtttggccatgggccccccttattatgaagcaatagcctcatcaggagaggtcgcctactccaccgaccttgaccggtgccgctgggggacccaaggaaagctcaccctcactgaggtctcaggacacgggttgtgcataggaaaggtgccctttacccatcagcatctctgcaatcagaccctatccatcaattcctccggagaccatcagtatctgctcccctccaaccatagctggtgggcttgcagcactggcctcaccccttgcctctccacctcagtttttaatcagactagagatttctgtatccaggtccagctgattcctcgcatctattactatcctgaagaagttttgttacaggcctatgacaattctcaccccaggactaaaagagaggctgtctcacttaccctagctgttttactggggttgggaatcacggcgggaataggtactggttcaactgccttaattaaaggacctatagacctccagcaaggcctgacaagcctccagatcgccatagatgctgacctccgggccctccaagactcagtcagcaagttagaggactcactgacttccctgtccgaggtagtgctccaaaataggagaggccttgacttgctgtttctaaaagaaggtggcctctgtgcggccctaaaggaagagtgctgtttttacatagaccactcaggtgcagtacgggactccatgaaaaaactcaaagaaaaactggataaaagacagttagagcgccagaaaagccaaaactggtatgaaggatggttcaataactccccttggttcactaccctgctatcaaccatcgctgggcccctattactcctccttctgttgctcatcctcgggccatgcatcatcaataagttagttcaattcatcaatgataggataagtgcagttaaaatttaa

SEQ ID NO: 8 - DNA, 2013 bp, Gibbon leukemia virus
accatggtcctgctgcctgggtctatgctgctgacttctaacctgcaccacctgcgacaccagatgtctcccggctcatggaaacggctgatcatcctgctgagctgcgtgttcggaggaggaggcacctccctgcagaacaagaatcctcaccagccaatgaccctgacatggcaggtgctgtcccagacaggcgacgtggtgtgggataccaaggcagtgcagccaccttggacatggtggcccaccctgaagcctgacgtgtgcgccctggccgcctccctggagtcttgggacatccccggcacagacgtgagcagcagcaagagggtgagaccacccgactctgattatacagccgcctacaagcagatcacctggggcgccatcggctgtagctatcctcgggcccgcacaaggatggccagctccaccttttacgtgtgcccacgcgacggaaggaccctgtctgaggcaaggagatgtggcggcctggagagcctgtattgcaaggagtgggattgtgagaccacaggcacaggctactggctgtctaagtctagcaaggacctgatcaccgtgaagtgggatcagaacagcgagtggacacagaagttccagcagtgccaccagaccggctggtgtaatcccctgaagatcgactttacagataagggcaagctgtccaaggactggatcaccggcaagacatggggcctgagattctacgtgtctggccaccctggcgtgcagtttacaatccggctgaagatcaccaacatgccagcagtggcagtgggaccagacctggtgctggtggagcagggacctccacgcacctccctggccctgccccctccactgccccctagggaggccccaccccctagcctgcccgattctaacagcacagccctggccacctccgcccagacccctacagtgcgcaagaccatcgtgacactgaataccccaccccctaccacaggcgacaggctgttcgatctggtgcagggcgcctttctgacactgaacgccaccaatcctggcgcaaccgagagctgctggctgtgcctggctatgggcccaccctactatgaggcaatcgcctcctctggagaggtggcatattccacagacctggatagatgcagatggggcacccagggcaagctgaccctgacagaggtgtctggccacggcctgtgcatcggcaaggtgccattcacacaccagcacctgtgcaaccagaccctgagcatcaatagctccggcgaccaccagtacctgctgccaagcaaccactcctggtgggcatgctccacaggactgaccccatgtctgagcaccagcgtgttcaaccagaccagagacttttgtatccaggtgcagctgatccctcggatctactattacccagaggaggtgctgctgcaggcctatgataattcccacccaagaacaaagagggaggccgtgtctctgaccctggccgtgctgctgggactgggaatcacagcaggaatcggcacaggcagcaccgccctgatcaagggaccaatcgacctgcagcagggactgacctccctgcagatcgccatcgacgccgatctgagagccctgcaggacagcgtgtccaagctggaggattctctgacctctctgagcgaggtggtgctgcagaacaggaggggcctggacctgctgttcctgaaggagggaggactgtgcgccgccctgaaggaggagtgctgtttttatatcgaccactctggcgccgtgcgggatagcatgaagaagctgaaggagaagctggataagcgccagctggagaggcagaagagccagaattggtacgagggctggttcaacaattccccctggtttaccacactgctgtctaccatcgcaggacctctgttattactgctgctgctgctgatcctgggcccatgtatcatcaacaagctggtgcagtttatcaacgaccgaatctccgcagtgaaaatctaa

SEQ ID NO: 9 - protein, 669 aa, Gibbon leukemia virus
MVLLPGSMLLTSNLHHLRHQMSPGSWKRLIILLSCVFGGGGTSLQNKNPHQPMTLTWQVLSQTGDVVWDTKAVQPPWTWWPTLKPDVCALAASLESWDIPGTDVSSSKRVRPPDSDYTAAYKQITWGAIGCSYPRARTRMASSTFYVCPRDGRTLSEARRCGGLESLYCKEWDCETTGTGYWLSKSSKDLITVKWDQNSEWTQKFQQCHQTGWCNPLKIDFTDKGKLSKDWITGKTWGLRFYVSGHPGVQFTIRLKITNMPAVAVGPDLVLVEQGPPRTSLALPPPLPPREAPPPSLPDSNSTALATSAQTPTVRKTIVTLNTPPPTTGDRLFDLVQGAFLTLNATNPGATESCWLCLAMGPPYYEAIASSGEVAYSTDLDRCRWGTQGKLTLTEVSGHGLCIGKVPFTHQHLCNQTLSINSSGDHQYLLPSNHSWWACSTGLTPCLSTSVFNQTRDFCIQVQLIPRIYYYPEEVLLQAYDNSHPRTKREAVSLTLAVLLGLGITAGIGTGSTALIKGPIDLQQGLTSLQIAIDADLRALQDSVSKLEDSLTSLSEVVLQNRRGLDLLFLKEGGLCAALKEECCFYIDHSGAVRDSMKKLKEKLDKRQLERQKSQNWYEGWFNNSPWFTTLLSTIAGPLLLLLLLLILGPCIINKLVQFINDRISAVKI

SEQ ID NO: 10 - DNA, 759 bp, Artificial Sequence
  Homo sapiens
atgatcgagacctacaatcagacaagcccacggtccgccgcaaccggactgcctatcagcatgaagatcttcatgtacctgctgaccgtgtttctgatcacacagatgatcggctccgccctgttcgccgtgtatctgcacaggagactggacaagatcgaggatgagcgcaatctgcacgaggacttcgtgtttatgaagaccatccagcggtgcaacacaggcgagaggagcctgtctctgctgaattgtgaggagatcaagtcccagttcgagggctttgtgaaggatatcatgctgaacaaggaggagacaaagaaggacgaggatccacagatcgcagcacacgtggtgtccgaggcaaactctaatgccgccagcgtgctgcagtgggccaagaagggctactataccatgaagtctaacctggtgacactggagaatggcaagcagctgaccgtgaagaggcagggcctgtactatatctatgcccaggtgacattctgctctaacagagaggcaagctcccaggcacccttcatcgtgggactgtggctgaagccctctagcggcagcgagaggatcctgctgaaggccgccaatacccactcctctagccagctgtgcgagcagcagtccatccacctgggaggcgtgttcgagctgcagcctggagccagcgtgttcgtgaacgtgacagacccatctcaggtgagccacggcaccggcttcacaagctttggcctgctgaagctgtga

SEQ ID NO: 11 - protein, 252 aa, Artificial Sequence
  Homo sapiens
MIETYNQTSPRSAATGLPISMKIFMYLLTVFLITQMIGSALFAVYLHRRLDKIEDERNLHEDFVFMKTIQRCNTGERSLSLLNCEEIKSQFEGFVKDIMLNKEETKKDEDPQIAAHVVSEANSNAASVLQWAKKGYYTMKSNLVTLENGKQLTVKRQGLYYIYAQVTFCSNREASSQAPFIVGLWLKPSSGSERILLKAANTHSSSQLCEQQSIHLGGVFELQPGASVFVNVTDPSQVSHGTGFTSFGLLKL

SEQ ID NO: 12 - DNA, 1416 bp, Homo sapiens
atgctgccctttctgagcatgctggtgctgctggtgcagcctctgggaaacctgggagccgagatgaagagcctgtcccagagatctgtgcctaacacctgcacactggtcatgtgcagccccaccgagaatggactgcctggaagggacggaagggatggaagggagggccctcggggcgagaagggcgacccaggactgcctggaccaatgggactgagcggactgcagggaccaacaggacctgtgggaccaaagggagagaacggatccgccggagagccaggccctaagggcgagaggggcctgtctggcccccctggcctgccaggcatcccaggccccgccggcaaggagggcccatccggcaagcagggcaatatcggcccccagggcaagcctggcccaaagggcgaggcaggaccaaagggagaagtgggagcacctggcatgcagggatccaccggagcaaagggatctacaggaccaaagggcgagcgcggcgccccaggcgtgcagggcgcccccggcaatgcaggagcagcaggaccagcaggacctgcaggcccacagggcgcccctggctctaggggcccacccggcctgaagggcgacaggggagtgcctggcgataggggcatcaagggagagagcggactgccagattccgccgccctgaggcagcagatggaggccctgaagggcaagctgcagaggctggaggtggccttctcccactaccagaaggccgccctgtttccagacggccacaggagactggacaagatcgaggatgagcgcaacctgcacgaggatttcgtgtttatgaagaccatccagagatgcaacacaggcgagcggtctctgagcctgctgaattgtgaggagatcaagtctcagttcgagggctttgtgaaggacatcatgctgaacaaggaggagaccaagaaggagaatagcttcgagatgcagaagggcgatcagaatccccagatcgcagcacacgtgatcagcgaggcaagctccaagaccacatccgtgctgcagtgggccgagaagggctactataccatgtccaacaatctggtgacactggagaacggcaagcagctgaccgtgaagagacagggcctgtactatatctatgcccaggtgacattctgctctaatcgggaggcctctagccaggccccttttatcgcctctctgtgcctgaagagcccaggcagattcgagcggatcctgctgagggccgccaacacccactcctctgccaagccatgcggacagcagagcatccacctgggaggcgtgttcgagctgcagccaggagcctccgtgtttgtgaatgtgacagacccatcccaggtgtctcacggaaccggcttcacatcctttggcctgctgaagctgtga

SEQ ID NO: 13 - protein, 471 aa, Homo sapiens
MLPFLSMLVLLVQPLGNLGAEMKSLSQRSVPNTCTLVMCSPTENGLPGRDGRDGREGPRGEKGDPGLPGPMGLSGLQGPTGPVGPKGENGSAGEPGPKGERGLSGPPGLPGIPGPAGKEGPSGKQGNIGPQGKPGPKGEAGPKGEVGAPGMQGSTGAKGSTGPKGERGAPGVQGAPGNAGAAGPAGPAGPQGAPGSRGPPGLKGDRGVPGDRGIKGESGLPDSAALRQQMEALKGKLQRLEVAFSHYQKAALFPDGHRRLDKIEDERNLHEDFVFMKTIQRCNTGERSLSLLNCEEIKSQFEGFVKDIMLNKEETKKENSFEMQKGDQNPQIAAHVISEASSKTTSVLQWAEKGYYTMSNNLVTLENGKQLTVKRQGLYYIYAQVTFCSNREASSQAPFIASLCLKSPGRFERILLRAANTHSSAKPCGQQSIHLGGVFELQPGASVFVNVTDPSQVSHGTGFTSFGLLKL

SEQ ID NO: 14 - DNA, 1412 bp, Mus musculus
atgctgcccttcctgagcatgctggtgctgctggtgcagcctctgggcaatctgggcgccgagatgaagtccctgtctcagaggagcgtgccaaacacctgcacactggtcatgtgctctccaaccgagaatggactgccaggaagggacggaagagatggaagggagggaccaaggggagagaagggcgaccctggactgcctggaccaatgggactgtccggactgcagggaccaacaggccctgtgggaccaaagggagagaatggaagcgccggagagccaggacctaagggagagaggggcctgtccggcccccctggcctgcctggcatcccaggccccgccggcaaggagggcccttctggcaagcagggcaacatcggaccacagggcaagcctggaccaaagggagaggcaggaccaaagggagaagtgggagcacccggcatgcagggcagcaccggagcaaagggatccaccggccctaagggagagagaggagcacctggagtgcagggcgccccaggcaatgcaggagcagcaggaccagcaggacctgcaggcccacagggcgccccaggcagccggggcccacccggcctgaagggcgacaggggagtgccaggcgataggggcatcaagggagagtccggactgccagactctgccgccctgaggcagcagatggaggccctgaagggcaagctgcagaggctggaggtggccttctcccactaccagaaggccgccctgtttccagacggacacaggagactggataaggtggaggaggaggtgaacctgcacgaggatttcgtgttcatcaagaagctgaagaggtgcaacaagggcgagggcagcctgtccctgctgaattgtgaggagatgcggcgccagttcgaggacctggtgaaggatatcaccctgaacaaggaggagaagaaggagaattcttttgagatgcagaggggcgacgaggatcctcagatcgcagcacacgtggtgtccgaggcaaactctaatgccgccagcgtgctgcagtgggccaagaagggctactataccatgaagtctaacctggtcatgctggagaatggcaagcagctgacagtgaagagagagggcctgtactacgtgtacacccaggtgacattctgcagcaacagagagcccagctcccagcggccttttatcgtgggcctgtggctgaagccctctatcggaagcgagaggatcctgctgaaggcagccaatacccactctagctcccagctgtgcgagcagcagtccgtgcacctgggaggcgtgttcgagctgcaggcaggagcaagcgtgttcgtgaacggacagaggccagccaggtcatccacagagtgggcttctctagctttggcctgctgaagctgtga

SEQ ID NO: 15 - protein, 470 aa, Mus musculus
MLPFLSMLVLLVQPLGNLGAEMKSLSQRSVPNTCTLVMCSPTENGLPGRDGRDGREGPRGEKGDPGLPGPMGLSGLQGPTGPVGPKGENGSAGEPGPKGERGLSGPPGLPGIPGPAGKEGPSGKQGNIGPQGKPGPKGEAGPKGEVGAPGMQGSTGAKGSTGPKGERGAPGVQGAPGNAGAAGPAGPAGPQGAPGSRGPPGLKGDRGVPGDRGIKGESGLPDSAALRQQMEALKGKLQRLEVAFSHYQKAALFPDGHRRLDKVEEEVNLHEDFVFIKKLKRCNKGEGSLSLLNCEEMRRQFEDLVKDITLNKEEKKENSFEMQRGDEDPQIAAHVVSEANSNAASVLQWAKKGYYTMKSNLVMLENGKQLTVKREGLYYVYTQVTFCSNREPSSQRPFIVGLWLKPSIGSERILLKAANTHSSSQLCEQQSVHLGGVFELQAGASVFVNVTEASQVIHRVGFSSFGLLKL

SEQ ID NO: 16 - DNA, 786 bp, Homo sapiens
atgatcgaaacatacaaccaaacttctccccgatctgcggccactggactgcccatcagcatgaaaatttttatgtatttacttactgtttttcttatcacccagatgattgggtcagcactttttgctgtgtatcttcatagaaggttggacaagatagaagatgaaaggaatcttcatgaagattttgtattcatgaaaacgatacagagatgcaacacaggagaaagatccttatccttactgaactgtgaggagattaaaagccagtttgaaggctttgtgaaggatataatgttaaacaaagaggagacgaagaaagaaaacagctttgaaatgcaaaaaggtgatcagaatcctcaaattgcggcacatgtcataagtgaggccagcagtaaaacaacatctgtgttacagtgggctgaaaaaggatactacaccatgagcaacaacttggtaaccctggaaaatgggaaacagctgaccgttaaaagacaaggactctattatatctatgcccaagtcaccttctgttccaatcgggaagcttcgagtcaagctccatttatagccagcctctgcctaaagtcccccggtagattcgagagaatcttactcagagctgcaaatacccacagttccgccaaaccttgcgggcaacaatccattcacttgggaggagtatttgaattgcaaccaggtgcttcggtgtttgtcaatgtgactgatccaagccaagtgagccatggcactggcttcacgtcctttggcttactcaaactctga

SEQ ID NO: 17 - protein, 261 aa, Homo sapiens
MIETYNQTSPRSAATGLPISMKIFMYLLTVFLITQMIGSALFAVYLHRRLDKIEDERNLHEDFVFMKTIQRCNTGERSLSLLNCEEIKSQFEGFVKDIMLNKEETKKENSFEMQKGDQNPQIAAHVISEASSKTTSVLQWAEKGYYTMSNNLVTLENGKQLTVKRQGLYYIYAQVTFCSNREASSQAPFIASLCLKSPGRFERILLRAANTHSSAKPCGQQSIHLGGVFELQPGASVFVNVTDPSQVSHGTGFTSFGLLKL

SEQ ID NO: 18 - DNA, 783 bp, Mus musculus
atgatagaaacatacagccaaccttcccccagatccgtggcaactggacttccagcgagcatgaagatttttatgtatttacttactgttttccttatcacccaaatgattggatctgtgctttttgctgtgtatcttcatagaagattggataaggtcgaagaggaagtaaaccttcatgaagattttgtattcataaaaaagctaaagagatgcaacaaaggagaaggatctttatccttgctgaactgtgaggagatgagaaggcaatttgaagaccttgtcaaggatataacgttaaacaaagaagagaaaaaagaaaacagctttgaaatgcaaagaggtgatgaggatcctcaaattgcagcacacgttgtaagcgaagccaacagtaatgcagcatccgttctacagtgggccaagaaaggatattataccatgaaaagcaacttggtaatgcttgaaaatgggaaacagctgacggttaaaagagaaggactctattatgtctacactcaagtcaccttctgctctaatcgggagccttcgagtcaacgcccattcatcgtcggcctctggctgaagcccagcagtggatctgagagaatcttactcaaggcggcaaatacccacagttcctcccagctttgcgagcagcagtctgttcacttgggcggagtgtttgaattacaagctggtgcttctgtgtttgtcaacgtgactgaagcaagccaagtgatccacagagttggcttctcatcttttggcttactcaaactctga

SEQ ID NO: 19 - protein, 260 aa, Mus musculus
MIETYSQPSPRSVATGLPASMKIFMYLLTVFLITQMIGSVLFAVYLHRRLDKVEEEVNLHEDFVFIKKLKRCNKGEGSLSLLNCEEMRRQFEDLVKDITLNKEEKKENSFEMQRGDEDPQIAAHVVSEANSNAASVLQWAKKGYYTMKSNLVMLENGKQLTVKREGLYYVYTQVTFCSNREPSSQRPFIVGLWLKPSSGSERILLKAANTHSSSQLCEQQSVHLGGVFELQAGASVFVNVTEASQVIHRVGFSSFGLLKL

SEQ ID NO: 20 - DNA, 930 bp, Mus musculus
atggatcagcacacactggacgtggaggataccgctgacgctaggcacccagctggcacctcctgcccttctgatgccgctctgctgcgcgacacaggactgctggccgatgccgctctgctgtctgacacagtgcggccaaccaacgccgctctgccaaccgatgctgcttaccctgctgtgaacgtgagggacagagaggctgcttggccacctgccctgaacttctgcagccgccaccctaagctgtacggcctggtggccctggtgctgctgctgctgatcgctgcttgcgtgccaatctttacccggacagagccacgccccgctctgacaatcaccacatcccccaacctgggcaccagggagaacaacgccgatcaggtgacaccagtgtctcacatcggctgccccaacaccacacagcagggaagcccagtgttcgccaagctgctggctaagaaccaggccagcctgtgcaacaccacactgaactggcacagccaggacggagctggaagctcctacctgtcccagggcctgagatacgaggaggataagaaggagctggtggtggactcccctggactgtactacgtgttcctggagctgaagctgtctccaacctttacaaacaccggccacaaggtgcagggatgggtgtctctggtgctgcaggctaagccccaggtggacgatttcgataacctggccctgaccgtggagctgtttccttgtagcatggagaacaagctggtggacaggtcttggagccagctgctgctgctgaaggctggccacaggctgtccgtgggactgagagcctacctgcacggcgcccaggatgcttacagagactgggagctgagctaccctaacaccacatccttcggactgtttctggtgaagcctgacaacccatgggagtga

SEQ ID NO: 21 - DNA, 765 bp, Homo sapiens
atggagtacgcctctgacgccagcctggatccagaggccccttggccacctgcaccaagggcccgcgcctgccgcgtgctgccctgggccctggtggccggcctgttattactgctgctgctggccgccgcctgcgccgtgttcctggcatgtccttgggccgtgagcggagccagagcctccccaggctctgccgccagccctcggctgagagagggaccagagctgtccccagacgatccagcaggcctgctggacctgaggcagggaatgtttgcccagctggtggcccagaacgtgctgctgatcgacggccccctgtcctggtactctgatcctggcctggccggcgtgtctctgaccggcggcctgagctataaggaggatacaaaggagctggtggtggccaaggccggcgtgtactacgtgttcttccagctggagctgaggagagtggtggcaggagagggctctggaagcgtgtccctggccctgcacctgcagcccctgcggagcgccgcaggagccgccgccctggccctgaccgtggacctgccaccagccagctccgaggcaaggaattccgccttcggctttcagggcagactgctgcacctgtctgccggacagaggctgggagtgcacctgcacaccgaggccagggcccgccacgcatggcagctgacccagggagcaacagtgctgggcctgttccgcgtgacacctgagatcccagcaggcctgcctagcccacggtccgagtga

SEQ ID NO: 22 - DNA, 1389 bp, Mus musculus
atgctgcctttcctgtccatgctggtgctgctggtgcagccactgggcaacctgggagccgagatgaagtctctgagccagcgcagcgtgcctaacacctgcacactggtcatgtgctcccctacagagaacggcctgccaggaagggacggaagagatggaagggagggaccaaggggagagaagggcgaccccggactgcctggaccaatgggactgagcggcctgcagggaccaaccggccccgtgggacctaagggagagaacggatccgctggagagccaggacctaagggagagagaggactgtctggaccacctggactgccaggaatcccaggaccagctggcaaggagggaccatccggcaagcagggaaacatcggaccacagggaaagcctggaccaaagggagaggctggacctaagggagaagtgggcgccccaggaatgcagggctctacaggagctaagggcagcaccggaccaaagggagagaggggagcccccggagtgcagggagcccctggcaacgctggagccgctggcccagccggacccgctggccctcagggagcccccggctctaggggaccaccaggcctgaagggagacagaggcgtgcccggagatcggggcatcaagggagagagcggcctgcctgactccgccgctctgagacagcagatggaggctctgaagggcaagctgcagcggctggaggtggccttctcccactaccagaaggccgctctgtttcctgacggaaggacagagcccaggcctgctctgaccatcaccacatctccaaacctgggcacaagagagaacaacgccgatcaggtgacccccgtgtctcacatcggatgccctaacaccacacagcagggcagccccgtgtttgccaagctgctggctaagaaccaggccagcctgtgcaacaccacactgaactggcactcccaggatggcgccggaagctcctacctgtctcagggcctgcggtacgaggaggacaagaaggagctggtggtggatagcccaggcctgtactacgtgttcctggagctgaagctgtcccccacctttacaaacaccggacacaaggtgcagggatgggtgagcctggtgctgcaggctaagccccaggtggacgatttcgacaacctggccctgaccgtggagctgtttccttgctctatggagaacaagctggtggatagatcctggagccagctgctgctgctgaaggctggacaccgcctgagcgtgggcctgagggcttacctgcacggagctcaggacgcttacagggattgggagctgtcctaccctaacaccacatctttcggcctgtttctggtgaagccagacaacccctgggagtga

SEQ ID NO: 23 - DNA, 1389 bp, Homo sapiens
atgctgctgttcctgctgtccgccctggtgctgctgacccagcctctgggctacctggaggccgagatgaagacctattctcaccggacaatgccaagcgcctgcacactggtcatgtgcagcagcgtggagtctggcctgccaggaagggacggaagggatggaagggagggacctagaggcgagaagggcgaccctggcctgccaggagcagcaggacaggcaggaatgcccggccaggccggccccgtgggacctaagggcgacaacggaagcgtgggagagccaggaccaaagggcgataccggcccttccggaccacctggaccaccaggcgtgcctggcccagccggcagggagggccctctgggcaagcagggcaatatcggcccacagggcaagcccggccctaagggcgaggccggccccaagggcgaagtgggcgcccctggcatgcagggaagcgccggagcccgcggcctggccggacctaagggcgagagaggcgtgcctggagagaggggcgtgccaggaaacacaggcgcagcaggatctgccggagcaatgggaccccagggcagccctggcgccaggggccctccaggcctgaagggcgacaagggcatcccaggcgataagggagcaaagggagagagcggcctgccagatgtggcctccctgcgccagcaggtggaggccctgcagggccaggtgcagcacctgcaggccgccttctctcagtacaagaaggtggagctgtttccaaacggcgcctgcccctgggccgtgagcggagcccgggcctccccaggctctgccgccagccctaggctgcgcgagggaccagagctgagcccagacgatccagcaggcctgctggacctgagacagggaatgttcgcccagctggtggcccagaatgtgctgctgatcgacggcccactgtcctggtactctgatccaggcctggccggcgtgtccctgaccggcggcctgtcttataaggaggatacaaaggagctggtggtggccaaggccggcgtgtactacgtgttcttccagctggagctgaggagagtggtggcaggagagggatccggatctgtgagcctggccctgcacctgcagcccctgcggtccgccgcaggagccgccgccctggccctgaccgtggacctgccacctgcctctagcgaggcacgcaattccgccttcggctttcagggccggctgctgcacctgtctgccggacagagactgggagtgcacctgcacaccgaggcccgggccagacacgcctggcagctgacccagggagcaacagtgctgggcctgtttagggtgacacctgagatcccagccggcctgccaagcccccgctccgagtga

SEQ ID NO: 24 - DNA, 522 bp, Mus musculus
atggaggagatgcctctgagggagagctccccacagagggccgagagatgcaagaagagctggctgctgtgcatcgtggctctgctgctgatgctgctgtgctctctgggcaccctgatctacacaagcctgaagccaaccgccatcgagtcctgtatggtgaagttcgagctgtctagctccaagtggcacatgacatcccccaagcctcactgcgtgaacaccacatctgacggaaagctgaagatcctgcagagcggcacctacctgatctacggacaggtcatccccgtggacaagaagtacatcaaggataacgcccctttcgtggtgcagatctacaagaagaacgacgtgctgcagacactgatgaacgattttcagatcctgcccatcggcggagtgtacgagctgcacgctggcgacaacatctacctgaagttcaactccaaggatcacatccagaagaccaacacatactggggaatcatcctgatgccagatctgccctttatctcttga

SEQ ID NO: 25 - DNA, 600 bp, Homo sapiens
atgaccctgcacccaagccccatcacatgcgagttcctgttttctaccgccctgatcagcccaaagatgtgcctgagccacctggagaatatgcccctgtcccactctcggacacagggagcccagagaagctcctggaagctgtggctgttctgctctatcgtgatgctgctgttcctgtgcagcttttcctggctgatcttcatctttctgcagctggagacagccaaggagccttgcatggccaagtttggccctctgccatccaagtggcagatggcctctagcgagcccccttgcgtgaacaaggtgagcgactggaagctggagatcctgcagaacggcctgtacctgatctatggccaggtggcccccaacgccaattacaacgacgtggcccctttcgaggtgcggctgtataagaacaaggatatgatccagaccctgacaaataagtctaagatccagaacgtgggcggcacatacgagctgcacgtgggcgacaccatcgacctgatcttcaacagcgagcaccaggtgctgaagaacaatacatattggggcatcatcctgctggccaacccccagtttatctcctga

SEQ ID NO: 26 - DNA, 1164 bp, Mus musculus
atgctgcctttcctgtctatgctggtgctgctggtgcagccactgggcaacctgggagccgagatgaagagcctgtcccagagatccgtgcccaacacctgcacactggtcatgtgctctcctaccgagaacggcctgccaggaagggacggaagagatggaagggagggacctcggggagagaagggcgacccaggactgcctggaccaatgggactgagcggcctgcagggaccaacaggccccgtgggacctaagggagagaacggaagcgccggagagccaggacctaagggagagaggggactgtccggaccacctggactgcctggaatcccaggaccagctggcaaggagggaccatccggcaagcagggaaacatcggaccacagggaaagcctggaccaaagggagaggctggaccaaagggagaagtgggcgctcctggaatgcagggctccaccggagccaagggctctacaggaccaaaaggagagaggggagctcccggagtgcagggagcccctggcaacgctggagccgctggcccagccggacccgctggccctcagggagccccaggcagcaggggaccacccggcctgaagggcgacaggggcgtgccaggagataggggcatcaagggagagtctggcctgccagacagcgccgctctgagacagcagatggaggccctgaagggcaagctgcagcggctggaggtggctttctcccactaccagaaggccgctctgtttccagatggcagcctgaagcccaccgccatcgagtcctgcatggtgaagtttgagctgagctcctctaagtggcacatgacatctcccaagcctcactgcgtgaacaccacatctgacggcaagctgaagatcctgcagagcggcacctacctgatctacggccaggtcatccccgtggacaagaagtacatcaaggataacgcccctttcgtggtgcagatctacaagaagaacgacgtgctgcagacactgatgaacgattttcagatcctgccaatcggcggagtgtacgagctgcacgctggcgacaacatctacctgaagttcaactctaaggatcacatccagaagaccaacacatactggggcatcatcctgatgccagatctgccctttatcagctga

SEQ ID NO: 27 - DNA, 1152 bp, Homo sapiens
atgctgctgttcctgctgtctgccctggtgctgctgacccagccactgggctacctggaggccgagatgaagacctattcccaccgcacaatgccttctgcctgcacactggtcatgtgcagcagcgtggagagcggcctgccaggaagggacggaagagatggaagggagggacccagaggcgagaagggcgaccctggcctgccaggagcagcaggacaggcaggaatgccaggccaggccggccccgtgggccctaagggcgacaatggatccgtgggagagccaggaccaaagggcgataccggcccttctggaccacctggaccaccaggcgtgcctggaccagcaggaagagagggacctctgggcaagcagggaaacatcggaccacagggcaagccaggccctaagggcgaggccggccccaagggcgaagtgggcgcccctggcatgcagggatccgccggagccaggggcctggccggacctaagggcgagcgcggcgtgcctggagagaggggcgtgccaggaaatacaggcgcagcaggatctgccggagcaatgggaccacagggcagccccggcgccagaggccctccaggcctgaagggcgacaagggaatccctggcgataagggagcaaagggagagagcggcctgccagacgtggcctccctgaggcagcaggtggaggccctgcagggacaggtgcagcacctgcaggccgccttcagccagtacaagaaggtggagctgtttccaaatggcgagacagccaaggagccctgcatggccaagttcggcccactgcccagcaagtggcagatggcctctagcgagcccccttgcgtgaacaaggtgagcgattggaagctggagatcctgcagaacggcctgtacctgatctatggccaggtggcccccaacgccaattacaacgacgtggccccttttgaggtgcggctgtataagaacaaggatatgatccagaccctgacaaataagtctaagatccagaacgtgggaggcacctacgagctgcacgtgggcgacacaatcgacctgatcttcaacagcgagcaccaggtgctgaagaacaatacatattggggcatcatcctgctggccaacccccagtttatctcctga

SEQ ID NO: 28 - DNA, 597 bp, Mus musculus
atggagggcgagggagtgcagcccctggatgagaacctggagaacggctcccggcctcgcttcaagtggaagaagaccctgcggctggtggtgtctggaatcaagggcgccggaatgctgctgtgctttatctacgtgtgcctgcagctgagctcctctcccgccaaggatccccctatccagaggctgagaggagctgtgaccaggtgcgaggacggacagctgttcatcagctcctacaagaacgagtaccagacaatggaggtgcagaacaacagcgtggtcatcaagtgtgatggcctgtacatcatctacctgaagggatccttctttcaggaggtgaagatcgacctgcactttcgggaggatcacaacccaatctctatccccatgctgaacgacggcaggagaatcgtgttcacagtggtggccagcctggcttttaaggacaaggtgtacctgaccgtgaacgccccagatacactgtgcgagcacctgcagatcaacgacggagagctgatcgtggtgcagctgacccctggctactgtgctccagagggatcttaccacagcacagtgaaccaggtgcccctgtga

SEQ ID NO: 29 - DNA, 552 bp, Homo sapiens
atggagagggtgcagcccctggaggagaacgtgggaaatgccgcccggcctagattcgagaggaacaagctgctgctggtggcctctgtgatccagggcctgggcctgctgctgtgcttcacctacatctgtctgcacttttctgccctgcaggtgagccacagatacccccgcatccagagcatcaaggtgcagttcaccgagtataagaaggagaagggctttatcctgacatcccagaaggaggacgagatcatgaaggtgcagaacaattctgtgatcatcaactgcgatggcttctacctgatctccctgaagggctatttttctcaggaagtgaatatcagcctgcactatcagaaggacgaggagccactgtttcagctgaagaaggtgcggagcgtgaattccctgatggtggccagcctgacctacaaggacaaggtgtatctgaacgtgaccacagataatacatccctggacgatttccacgtgaacggcggcgagctgatcctgatccaccagaatcccggcgagttttgcgtgctgtga

SEQ ID NO: 30 - DNA, 1215 bp, Mus musculus
atgctgcccttcctgtccatgctggtgctgctggtgcagcctctgggcaacctgggagccgagatgaagtctctgagccagagatccgtgccaaacacctgcacactggtcatgtgctctcccaccgagaacggcctgcctggaagggacggaagagatggaagggagggaccccggggagagaagggcgatcctggactgccaggacctatgggactgagcggcctgcagggaccaacaggccccgtgggacctaagggagagaacggaagcgccggagagccaggaccaaagggagagaggggactgtccggcccacctggactgcctggaatccctggaccagctggcaaggagggaccttccggcaagcagggaaacatcggaccacagggaaagccaggacctaagggagaggctggaccaaagggagaagtgggcgctcccggaatgcagggctctaccggagccaagggcagcacaggacctaagggagagaggggagctccaggagtgcagggagcccccggcaacgctggagctgctggaccagctggaccagctggccctcagggagccccaggctctaggggaccaccaggcctgaagggcgacaggggcgtgccaggagataggggcatcaagggagagagcggcctgccagattccgccgctctgagacagcagatggaggccctgaagggcaagctgcagcggctggaggtggctttcagccactaccagaaggccgctctgtttcctgacggcagctcctctccagccaaggatcctccaatccagcggctgcgcggagctgtgaccaggtgcgaggatggccagctgttcatcagctcctacaagaacgagtaccagacaatggaggtgcagaacaactctgtggtcatcaagtgtgacggcctgtacatcatctacctgaagggcagcttctttcaggaggtgaagatcgacctgcactttagagaggatcacaacccaatctccatccccatgctgaacgacggcaggagaatcgtgttcaccgtggtggcctctctggcttttaaggacaaggtgtacctgaccgtgaacgcccccgatacactgtgcgagcacctgcagatcaacgacggcgagctgatcgtggtgcagctgacccctggatactgtgctccagagggctcctaccactctacagtgaaccaggtgcctctgtga

SEQ ID NO: 31 - DNA, 1170 bp, Homo sapiens
atgctgctgttcctgctgagcgccctggtgctgctgacccagccactgggctacctggaggccgagatgaagacctattcccacagaacaatgccttctgcctgcacactggtcatgtgcagcagcgtggagtccggcctgccaggaagggacggcagagatggcagggagggccccaggggcgagaagggcgaccccggcctgcctggagcagcaggccaggccggcatgccaggccaggccggcccagtgggccccaagggcgacaacggcagcgtgggcgagcccggccctaagggcgataccggcccctccggcccccctggcccacccggcgtgccaggaccagcaggaagggagggaccactgggcaagcagggcaatatcggacctcagggcaagcctggaccaaagggagaggcaggaccaaagggagaagtgggcgcccctggcatgcagggatctgccggagcccggggcctggccggccccaagggcgagagaggcgtgcccggcgagaggggcgtgcctggcaacacaggcgccgccggctccgccggcgccatgggacctcagggctctccaggagccagaggccctccaggcctgaagggcgacaagggaatccctggcgataagggagcaaagggagagagcggcctgccagacgtggcctccctgcggcagcaggtggaggccctgcagggccaggtgcagcacctgcaggccgccttcagccagtacaagaaggtggagctgtttcctaatggcgtgtctcaccgctacccacggatccagagcatcaaggtgcagttcaccgagtataagaaggagaagggctttatcctgacatctcagaaggaggacgagatcatgaaggtgcagaacaatagcgtgatcatcaactgcgatggcttctacctgatcagcctgaagggctatttttcccaggaagtgaatatctctctgcactatcagaaggatgaggagcctctgtttcagctgaagaaggtgagatctgtgaacagcctgatggtggcctccctgacctacaaggacaaggtgtatctgaacgtgaccacagataatacatctctggacgatttccacgtgaacggcggcgagctgatcctgatccaccagaatcccggcgagttttgcgtgctgtga

SEQ ID NO: 32 - DNA, 969 bp, Mus musculus
atgcagctgaagtgtccatgcttcgtgtccctgggaacaagacagcccgtctggaagaaactgcacgtgagctccggcttctttagcggcctggggctgtttctgctgctgctgtctagtctgtgcgccgcttccgcagagactgaagtcggagccatggtgggcagtaacgtggtcctgtcatgcatcgacccacaccgacggcatttcaacctgtctggcctgtacgtgtattggcagattgagaatcccgaagtgtcagtcacctactatctgccttacaagagcccagggatcaacgtggactcaagctataaaaatagggggcacctgtccctggattctatgaagcagggaaacttcagcctgtacctgaaaaatgtgacccctcaggacacacaggagttcacttgtcgcgtctttatgaacactgcaaccgaactggtgaagattctggaggaagtggtccggctgagagtcgcagccaactttagcactcctgtgatctctaccagtgattcctctaatccaggccaggagcggacatatacttgcatgtctaagaacggataccccgaacctaatctgtattggatcaacaccacagacaatagtctgattgataccgctctgcagaacaatacagtctacctgaacaagctggggctgtatgacgtgatctctactctgcggctgccatggaccagtagaggagatgtgctgtgctgcgtggagaacgtggccctgcaccagaatatcacctcaattagccaggctgagtcctttaccggcaacaatacaaagaatcctcaggagacacataacaatgaactgaaagtgctggtgccagtgctggccgtcctggctgcagcagctttcgtgtcttttatcatctacagaaggacccgccctcaccgctcatacactggacctaagaccgtgcagctggaactgacagaccatgcttga

SEQ ID NO: 33 - DNA, 909 bp, Homo sapiens
atgcgtctgggttcacctggtctgctgtttctgctgttttcaagtctgcgtgctgatactcaggagaaggaagtccgggctatggtcggaagtgacgtggagctgtcatgcgcttgtcccgaagggtcccggttcgacctgaacgatgtctacgtgtattggcagacctctgagagtaagaccgtggtcacataccacatccctcagaactccagcctggaaaatgtggattcaaggtatcggaacagagccctgatgtcccctgctggcatgctgcggggagacttctctctgagactgtttaatgtgacaccacaggatgagcagaaattccattgcctggtcctgtcacagtccctgggatttcaggaggtgctgagtgtcgaagtgactctgcacgtcgccgctaatttctccgtgcctgtggtcagcgcaccacatagcccctctcaggacgagctgacctttacatgtacttccatcaacggctacccccgccctaacgtgtactggattaacaagactgacaatagcctgctggatcaggcactgcagaacgacaccgtgtttctgaatatgcgaggactgtacgatgtggtcagcgtcctgcgtattgccaggaccccatctgtgaacatcgggtgctgtattgagaacgtcctgctgcagcagaatctgacagtggggagccagactggtaatgacatcggcgagagggataagattaccgaaaaccccgtgagtacaggcgagaagaacgcagccacatggtcaatcctggctgtgctgtgcctgctggtggtcgtggctgtcgcaattggctgggtgtgccgcgatcggtgtctgcagcactcttatgccggtgcttgggcagtgagtccagagactgaactgaccggccatgtctaa

SEQ ID NO: 34 - DNA, 1574 bp, Mus musculus
cttaagatggaaactgatactctgctgctctgggtgctgctcctctgggtgcctggttcaactggggacattcgacgggctgacattgtgatgacccagaccacactgagcctgcccgtgtccctgggcgaccaggccagcatctcctgccggagctcccagtctatcgtgcacagcaacggaaacacatacctggagtggtatctgcagaagcctggccagtccccaaagctgctgatctacaaggtgtccaacaggttcagcggcgtgcctgaccgcttttctggaagcggctccggaacagatttcaccctgaagatcagcagggtggaggctgaggacctgggcgtgtactactgcttccagggatcccacgtgccttacacctttggcggaggcacaaagctggagatcaagagagccgatgctgctccaaccgtgtctggaagcggaggcgggggttctggaggcggtgggagcggtggcggagggtctgaggctaagctgcaggagagcggccccgtgctggtgaagcctggagccagcgtgaagatgtcctgtaaggcttctggatacaccttcacagactactacatgaactgggtgaagcagagccacggcaagtccctggagtggatcggagtgatcaacccttacaacggcgacacctcttacaaccagaagtttaagggcaaggccaccctgacagtggataagtctagctccaccgcttacatggagctgaacagcctgacatccgaggattctgccgtgtactactgtgctaggtactacggaagctggttcgcctactggggccagggaacactgatcaccgtgtccacagccaagaccacaccccctagcgtgtaccccctggctcctaggtctagcagaggctgcaagccatgcatctgtaccgtgcccgaggtgagcagcgtgttcatctttccacccaagcccaaggacgtgctgaccatcacactgacccctaaggtgacatgcgtggtggtggatatcagcaaggacgatccagaggtgcagttctcctggtttgtggacgatgtggaggtgcacaccgcccagacacagccaagggaggagcagttcaactccacctttagatccgtgtctgagctgcccatcatgcaccaggactggctgaacggaaaggagttcaagtgccgggtgaactccgccgcttttcctgctccaatcgagaagaccatctctaagacaaagggccgcccaaaggctccacaggtgtacaccatccctccacccaaggagcagatggctaaggataaggtgagcctgacctgtatgatcacagacttctttcccgaggatatcacagtggagtggcagtggaacggacagcctgccgagaactacaagaacacccagccaatcatggacacagatggctcttacttcgtgtacagcaagctgaacgtgcagaagtctaactgggaggctggcaacaccttcacctgcagcgtgctgcacgaaggtctccataatcaccacaccgaaaagagcctcagtcacagccctgggaaatgaggcgcgcc

SEQ ID NO: 35 - DNA, 1484 bp, Homo sapiens
cttaagatggaaactgacaccctgctgctgtgggtcctgctgctgtgggtgcctggatccaccggcgatatcgtgctgacccagtctcctggcacactgagtctgtcaccaggggagcgagcaacactgtcttgtagagccagccagtctgtgggaagctcctacctggcttggtatcagcagaagccaggccaggcacccaggctgctgatctacggagccttcagccgggccactggcattccagacaggttctctggaagtggctcagggaccgacttcaccctgaccatcagccgactggagcccgaagacttcgccgtgtactattgccagcagtacggctctagtccttggacttttggacagggcaccaaagtggagatcaagcgcggcgggggaggctctgggggaggcgggagtggaggcgggggatcacaggtccagctggtggaaagcggcgggggagtggtccagccaggccggagcctgcggctgagctgcgccgcttcaggattcacattttcaagctataccatgcactgggtccggcaggcaccagggaagggactggagtgggtgaccttcatcagctatgacggcaacaacaagtattacgctgattccgtgaaagggaggtttaccattagccgcgacaactccaaaaatacactgtacctgcagatgaacagcctgcgggccgaggatactgctatctactattgcgcaagaaccgggtggctgggacccttcgactattggggccaggggactctggtcaccgtgtcctctgataagacacacacatgccctccctgtcctgcaccagagctgctgggcgggccatccgtgttcctgtttccacccaagcctaaagacaccctgatgatcagccggacacctgaagtcacttgcgtggtcgtggacgtgagtcacgaggatccagaagtcaagtttaactggtacgtggatggcgtcgaggtgcataatgccaagaccaaacctcgcgaggaacagtacaatagcacatatcgagtcgtgtccgtcctgactgtgctgcatcaggattggctgaacggcaaagagtataagtgcaaagtgagcaataaggcactgcctgccccaatcgagaaaacaatttccaaggctaaaggccagcccagggaacctcaggtgtacactctgcctccaagtcgcgaggaaatgaccaagaaccaggtgagcctgacctgtctggtgaaagggttctatccatcagacattgcagtggagtgggaaagcaatggacagcccgaaaacaattacaagaccacaccccctgtgctggacagcgatggctccttctttctgtattctaagctgactgtggataaaagtcgctggcagcaggggaacgtctttagctgttccgtgatgcatgaggctctgcacaatcattacacacagaagtctctgagtctgtcacccggcaaatgaggcgcgcc

SEQ ID NO: 36 - DNA, 632 bp, Artificial Sequence
  CMV promoter
gttgacattgattattgactagttattaatagtaatcaattacggggtcattagttcatagcccatatatggagttccgcgttacataacttacggtaaatggcccgcctggctgaccgcccaacgacccccgcccattgacgtcaataatgacgtatgttcccatagtaacgccaatagggactttccattgacgtcaatgggtggagtatttacggtaaactgcccacttggcagtacatcaagtgtatcatatgccaagtacgccccctattgacgtcaatgacggtaaatggcccgcctggcattatgcccagtacatgaccttatgggactttcctacttggcagtacatctacgtattagtcatcgctattaccatggtgatgcggttttggcagtacatcaatgggcgtggatagcggtttgactcacggggatttccaagtctccaccccattgacgtcaatgggagtttgttttggcaccaaaatcaacgggactttccaaaatgtcgtaacaactccgccccattgacgcaaatgggcggtaggcgtgtacggtgggaggtctatataagcagagctctctggctaactagagaacccactgcttactggcttatcgaaatt

SEQ ID NO: 37 - DNA, 394 bp, Artificial Sequence
  RSV promoter
tgtacgggccagatatacgcgtatctgaggggactagggtgtgtttaggcgaaaagcggggcttcggttgtacgcggttaggagtcccctcaggatatagtagtttcgcttttgcatagggagggggaaatgtagtcttatgcaatacacttgtagtcttgcaacatggtaacgatgagttagcaacatgccttacaaggagagaaaaagcaccgtgcatgccgattggtggaagtaaggtggtacgatcgtgccttattaggaaggcaacagacaggtctgacatggattggacgaaccactgaattccgcattgcagagataattgtatttaagtgcctagctcgatacaataaacgccatttgaccattcaccacattggtgtgcacctcc

SEQ ID NO: 38 - DNA, 188 bp, Artificial Sequence
  BGH polyA
ctgtgccttctagttgccagccatctgttgtttgcccctcccccgtgccttccttgaccctggaaggtgccactcccactgtcctttcctaataaaatgaggaaattgcatcgcattgtctgagtaggtgtcattctattctggggggtggggtggggcaggacagcaagggggaggattgggaagac

SEQ ID NO: 39 - DNA, 249 bp, Artificial Sequence
  SV40 late polyA
gacatgataagatacattgatgagtttggacaaaccacaactagaatgcagtgaaaaaaatgctttatttgtgaaatttgtgatgctattgctttatttgtgaaatttgtgatgctattgctttatttgtaaccattataagctgcaataaacaagttaacaacaacaattgcattcattttatgtttcaggttcagggggaggtgtgggaggttttttaaagcaagtaaaacctctacaaatgtggta

SEQ ID NO: 40 - DNA, 345 bp, Artificial Sequence
  SV40 enhancer promoter
gctgtggaatgtgtgtcagttagggtgtggaaagtccccaggctccccagcaggcagaagtatgcaaagcatgcatctcaattagtcagcaaccaggtgtggaaagtccccaggctccccagcaggcagaagtatgcaaagcatgcatctcaattagtcagcaaccatagtcccgcccctaactccgcccatcccgcccctaactccgcccagttccgcccattctccgccccatggctgactaattttttttatttatgcagaggccgaggccgcctcggcctctgagctattccagaagtagtgaggaggcttttttggaggcctaggcttttgcaaaaagct

SEQ ID NO: 41 - DNA, 99 bp, Artificial Sequence
  Rabbit beta-globin polyA
gacctctggctaataaaggaaatttattttcattgcaatagtgtgttggaattttttgtgtctctcactcggaaggacatatgggagggcaaatcattt

SEQ ID NO: 42 - DNA, 723 bp, Artificial Sequence
  GFP
accatggtgagcaagggcgaggagctgttcaccggggtggtgcccatcctggtcgagctggacggcgacgtaaacggccacaagttcagcgtgtccggcgagggcgagggcgatgccacctacggcaagctgaccctgaagttcatctgcaccaccggcaagctgcccgtgccctggcccaccctcgtgaccaccctgacctacggcgtgcagtgcttcagccgctaccccgaccacatgaagcagcacgacttcttcaagtccgccatgcccgaaggctacgtccaggagcgcaccatcttcttcaaggacgacggcaactacaagacccgcgccgaggtgaagttcgagggcgacaccctggtgaaccgcatcgagctgaagggcatcgacttcaaggaggacggcaacatcctggggcacaagctggagtacaactacaacagccacaacgtctatatcatggccgacaagcagaagaacggcatcaaggtgaacttcaagatccgccacaacatcgaggacggcagcgtgcagctcgccgaccactaccagcagaacacccccatcggcgacggccccgtgctgctgcccgacaaccactacctgagcacccagtccgccctgagcaaagaccccaacgagaagcgcgatcacatggtcctgctggagttcgtgaccgccgccgggatcactctcggcatggacgagctgtacaagtaa

SEQ ID NO: 43 - DNA, 454 bp, Artificial Sequence
  MoMuLV LTR
ttaattaagtaacgccattttgcaaggcatggaaaaatacataactgagaatagagaagttcagatcaaggtcaggaacagatggaacagctgaatatgggccaaacaggatatctgtggtaagcagttcctgccccggctcagggccaagaacagatggaacagctgaatatgggccaaacaggatatctgtggtaagcagttcctgccccggctcagggccaagaacagatggtccccagatgcggtccagccctcagcagtttctagagaaccatcagatgtttccagggtgccccaaggacctgaaatgaccctgtgccttatttgaactaaccaatcagttcgcttctcgcttctgttcgcgcgcttctgctccccgagctcaataaaagagcccacaacccctcactcggggcgccagtcctccgattgactgagtcgcccgcttaag

SEQ ID NO: 44 - DNA, 1349 bp, Artificial Sequence
  EF1alpha promoter
ttaattaagagtaattcatacaaaaggactcgcccctgccttggggaatcccagggaccgtcgttaaactcccactaacgtagaacccagagatcgctgcgttcccgccccctcacccgcccgctctcgtcatcactgaggtggagaagagcatgcgtgaggctccggtgcccgtcagtgggcagagcgcacatcgcccacagtccccgagaagttggggggaggggtcggcaattgaaccggtgcctagagaaggtggcgcggggtaaactgggaaagtgatgtcgtgtactggctccgcctttttcccgagggtgggggagaaccgtatataagtgcagtagtcgccgtgaacgttctttttcgcaacgggtttgccgccagaacacaggtaagtgccgtgtgtggttcccgcgggcctggcctctttacgggttatggcccttgcgtgccttgaattacttccacgcccctggctgcagtacgtgattcttgatcccgagcttcgggttggaagtgggtgggagagttcgaggccttgcggttaaggagccccttcgcctcgtgcttgagttgaggcctggcttgggcgctggggccgccgcgtgcgaatctggtggcaccttcgcgcctgtctcgctgctttcgataagtctctagccatttaaaatttttgatgacctgctgcgacgctttttttctggcaagatagtcttgtaaatgcgggccaagatctgcacactggtatttcggtttttggggccgcgggcggcgacggggcccgtgcgtcccagcgcacatgttcggcgaggcggggcctgcgagcgcggccaccgagaatcggacgggggtagtctcaagctggccggcctgctctggtgcctggcctcgcgccgccgtgtatcgccccgccctgggcggcaaggctggcccggtcggcaccagttgcgtgagcggaaagatggccgcttcccggccctgctgcagggagctcaaaatggaggacgcggcgctcgggagagcgggcgggtgagtcacccacacaaaggaaaagggcctttccgtcctcagccgtcgcttcatgtgactccacggagtaccgggcgccgtccaggcacctcgattagttctcgagcttttggagtacgtcgtctttaggttggggggaggggttttatgcgatggagtttccccacactgagtgggtggagactgaagttaggccagcttggcacttgatgtaattctccttggaatttgccctttttgagtttggatcttggttcattctcaagcctcagacagtggttcaaagtttttttcttccatttcaggtgtcgtgacttaag

SEQ ID NO: 45 - DNA, 481 bp, Artificial Sequence
  HGH polyA
gacgggtggcatccctgtgacccctccccagtgcctctcctggccctggaagttgccactccagtgcccaccagccttgtcctaataaaattaagttgcatcattttgtctgactaggtgtccttctataatattatggggtggaggggggtggtatggagcaaggggcaagttgggaagacaacctgtagggcctgcggggtctattgggaaccaagctggagtgcagtggcacaatcttggctcactgcaatctccgcctcctgggttcaagcgattctcctgcctcagcctcccgagttgttgggattccaggcatgcatgaccaggctcagctaatttttgtttttttggtagagacggggtttcaccatattggccaggctggtctccaactcctaatctcaggtgatctacccaccttggcctcccaaattgctgggattacaggcgtgaaccactgctcccttccctgtccttt